European Patent Specification EP 3 434 761 B1, published January 18, 2023. Title: Method for Inducing Mesoderm with Increased Capacity for Differentiation into Blood Cell. Applicant: Megakaryon Corporation Kyoto University. Application Not yet assigned. The sequence listing filed with the application follows.

SEQUENCE LISTING (16 sequences)

SEQ ID NO: 1 - DNA, 20 bp, Artificial Sequence
  Forward primer for Beta-actin (ACTB)
tcctccctggagaagagcta

SEQ ID NO: 2 - DNA, 18 bp, Artificial Sequence
  Reverse primer for Beta-actin (ACTB)
cgtggatgccacaggact

SEQ ID NO: 3 - DNA, 20 bp, Artificial Sequence
  Forward primer for NANOG
atgcctcacacggagactgt

SEQ ID NO: 4 - DNA, 20 bp, Artificial Sequence
  Reverse primer for NANOG
cagggctgtcctgaataagc

SEQ ID NO: 5 - DNA, 23 bp, Artificial Sequence
  Forward primer for OCT3/4 (POU5F1)
gcttcaagaacatgtgtaagctg

SEQ ID NO: 6 - DNA, 19 bp, Artificial Sequence
  Reverse primer for OCT3/4 (POU5F1)
cacgagggtttctgctttg

SEQ ID NO: 7 - DNA, 20 bp, Artificial Sequence
  Forward primer for T
gctgtgacaggtacccaacc

SEQ ID NO: 8 - DNA, 21 bp, Artificial Sequence
  Reverse primer for T
catgcaggtgagttgtcagaa

SEQ ID NO: 9 - DNA, 18 bp, Artificial Sequence
  Forward primer for APJ
ggcagttctttgggtgct

SEQ ID NO: 10 - DNA, 20 bp, Artificial Sequence
  Reverse primer for APJ
gtggtgcgtaacaccatgac

SEQ ID NO: 11 - DNA, 20 bp, Artificial Sequence
  Forward primer for ETV2
gtggtgcgtaacaccatgac

SEQ ID NO: 12 - DNA, 22 bp, Artificial Sequence
  Reverse primer for ETV2
aaggccttctgaatgttctctg

SEQ ID NO: 13 - DNA, 22 bp, Artificial Sequence
  Forward primer for KDR
aaggccttctgaatgttctctg

SEQ ID NO: 14 - DNA, 23 bp, Artificial Sequence
  Reverse primer for KDR
cggaagaacaatgtagtctttgc

SEQ ID NO: 15 - DNA, 18 bp, Artificial Sequence
  Forward primer for RUNX1
acaaacccaccgcaagtc

SEQ ID NO: 16 - DNA, 23 bp, Artificial Sequence
  Reverse primer for RUNX1
catctagtttctgccgatgtctt